European Patent Application EP 4 151 730 A1, published March 22, 2023. Title: TREATMENT OF COVID-19 WITH REVERSE MICELLE SYSTEM COMPRISING UNMODIFIED OLIGONUCLEOTIDES. Applicant: MEDESIS PHARMA et al. The sequence listing filed with the application follows.

SEQUENCE LISTING (10 sequences)

SEQ ID NO: 1 - RNA, 22 nt, Artificial Sequence
  guide strand of siRNA A
uauagcuaaagacacgaaccgc

SEQ ID NO: 2 - RNA, 22 nt, Artificial Sequence
  passenger strand of siRNA B
gguucgugucuuuaguuauucu

SEQ ID NO: 3 - RNA, 22 nt, Artificial Sequence
  guide strand of siRNA B
uaaacuacaaauggaacaccac

SEQ ID NO: 4 - RNA, 22 nt, Artificial Sequence
  passenger strand of siRNA B
gguguucuauuuguaguuuucu

SEQ ID NO: 5 - RNA, 22 nt, Artificial Sequence
  guide strand of siRNA C
uugagugcaucauuauccaacc

SEQ ID NO: 6 - RNA, 22 nt, Artificial Sequence
  passenger strand of siRNA C
uuggauaaugaugcacucuucu

SEQ ID NO: 7 - RNA, 22 nt, Artificial Sequence
  guide strand of siRNA D
uuagcuaaagacacgaaccguc

SEQ ID NO: 8 - RNA, 22 nt, Artificial Sequence
  passenger strand of siRNA D
cgguucgugucuuuaguuaucu

SEQ ID NO: 9 - RNA, 21 nt, Artificial Sequence
  guide strand of siRNA E
uuugagugcaucauuauccac

SEQ ID NO: 10 - RNA, 21 nt, Artificial Sequence
  passenger strand of siRNA E
ggauaaugaugcacuuaaucu